European Patent Application EP 4 151 231 A1, published March 22, 2023. Title: ANTIBODY THERAPEUTICS THAT BIND CTLA4. Applicant: SORRENTO THERAPEUTICS, INC. Application EP, filed February 12, 2016. The sequence listing filed with the application follows.

SEQUENCE LISTING (46 sequences)

SEQ ID NO: 1 - protein, 114 aa, synthetic construct
  REGION 1..114: note = Description of Artificial Sequence: Syntheticpolypeptide
EVQLVQSGGGLVQPGRSLRLSCRGSNFNFDDLAISWVRQAPGKGLEWLGFVRSKAYGETTDYVASVKGRFTISRDDSKFIAWLQMDSLKTDDTAVYYCTTFNYWGQGTLVTVSS

SEQ ID NO: 2 - protein, 108 aa, synthetic construct
  REGION 1..108: note = Description of Artificial Sequence: Syntheticpolypeptide
LPVLTQPPSVSVAPGKTARISCGGNNIASEAVHWYQKKPGQAPVLVIYYDSDRPSGIPERFSGSNSGNTATLRISRVDAGDEADYYCQVWDRTTDQPVFGGGTKLTVL

SEQ ID NO: 3 - protein, 119 aa, synthetic construct
  REGION 1..119: note = Description of Artificial Sequence: Syntheticpolypeptide
QMQLVQSGAEVKMPGSSVRISCKASGGSFTTHFINWVRQAPGQGLEWMGWMNPNTGNTGYAERFQGRVTLTRDTSISTAYLELSSLRSDDTAVYYCARNPAESGRFDPWGQGTLVTVSS

SEQ ID NO: 4 - protein, 111 aa, synthetic construct
  REGION 1..111: note = Description of Artificial Sequence: Syntheticpolypeptide
QSALTQPPSASGSPGRSVTISCTGTSNNVGGYNYVSWYQQHPGKAPKLMIYEVTKRPSGVPDRFSGSKSGNTASLTVSGLQAEDEADYYCGTWDGSLNAYVFGTGTKVTVL

SEQ ID NO: 5 - protein, 119 aa, synthetic construct
  REGION 1..119: note = Description of Artificial Sequence: Syntheticpolypeptide
QVQLVESGGGLIQPGGSLRLSCAASGFSVSNNYMNWVRQAPGKGLEWVSVIYRGGSTYYADSVKGRFTISRDNSKNTLYLQMNSLRTEDTAVYYCLREGGTSGDYVNDWGQGTLVTVSS

SEQ ID NO: 6 - protein, 110 aa, synthetic construct
  REGION 1..110: note = Description of Artificial Sequence: Syntheticpolypeptide
QSVVTQPPSVSGAPGQRVTISCTGSSSNIGAGYDVHWYQQLPGTAPKLLIYGNKNRPSGVPDRFSGSKSGTSASLAITGLQAEDEADYYCQAYDSSLSVVFGGGTKLTVL

SEQ ID NO: 7 - protein, 124 aa, synthetic construct
  REGION 1..124: note = Description of Artificial Sequence: Syntheticpolypeptide
QMQLVQSGAEVKKPGASVKVSCKASGGTFSSYAISWVRQAPGQGLEWMGGIIPIFGTANYAQKFQGRVTITADESTSTAYMELSSLRSEDTAVYYCAREIGSYSSGWYRAFDIWGQGTMVTVSS

SEQ ID NO: 8 - protein, 107 aa, synthetic construct
  REGION 1..107: note = Description of Artificial Sequence: Syntheticpolypeptide
DIVMTQSPSTLSASVGDRVTITCRASQSISSWLAWYQQKPGKAPQLLIYKASNLQSGVPSRFSGSGSVTEFSLTISSLLPEDFATYYCQQYSRPPWTFGQGTKVEIK

SEQ ID NO: 9 - protein, 124 aa, synthetic construct
  REGION 1..124: note = Description of Artificial Sequence: Syntheticpolypeptide
QVQLVESGGGLVQPGGSLRLSCAASGFTFSNYAMNWVRQTPGKGLEWVSVNYNDGFGTFNGYYADSVKGRFIISRDNSKNTLYLQMNSLRVDDTAVYYCARDSGVAGPYYFDNWGQGTLVTVSS

SEQ ID NO: 10 - protein, 107 aa, synthetic construct
  REGION 1..107: note = Description of Artificial Sequence: Syntheticpolypeptide
AIQLTQSPSTLSASVGDRVTITCRASQSISSWLAWYQQKPGKAPKLLIYKASSLESGVPSRFSGSGSGTEFTLTISSLQPDDFATYYCQQYNSSPLTFGGGTKLEIK

SEQ ID NO: 11 - protein, 125 aa, synthetic construct
  REGION 1..125: note = Description of Artificial Sequence: Syntheticpolypeptide
QVQLVQSGAEVKKPGATVKVSCTASGFPFRNYAMHWVRQAPGQRLEWLGWIDAGNGNTKYSQTFHGRVTITRDTSASTAYMELSSLRSEDTAVYYCARDLLWPYLVTSGGAFDIWGQGTMVTVSS

SEQ ID NO: 12 - protein, 110 aa, synthetic construct
  REGION 1..110: note = Description of Artificial Sequence: Syntheticpolypeptide
SYELMQPPSTSGTPGQRVTISCSGSSSNIGSHIVNWYQQFPGAAPQLLIYNDDQRPSGVPDRFSGSKSGASASLAISGLQSEDEAHYYCSAWDDILKGPVFGGGTKLTVL

SEQ ID NO: 13 - protein, 118 aa, synthetic construct
  REGION 1..118: note = Description of Artificial Sequence: Syntheticpolypeptide
QVQLVQSGAEVKKPGASVKVSCKASGYTFTTHYIHWVRQAPGQGLEWMAIINPNDGVKVYAQKFKGRLTVASDTSATTVYMDLSGLTSDDTAVYYCGREQHGGHHDYWGQGTLVTVSS

SEQ ID NO: 14 - protein, 111 aa, synthetic construct
  REGION 1..111: note = Description of Artificial Sequence: Syntheticpolypeptide
QAGLTQPASVSGSPGQSITISCTGTSSDVGGYNYVSWYQQHPGKAPKLMIYDVTNRPSGVSNRFSGSKSGNTASLTISGLQAEDEADYYCKSYTSSSTPYVFGTGTKVTVL

SEQ ID NO: 15 - protein, 114 aa, synthetic construct; identical to SEQ ID NO: 1
  REGION 1..114: note = Description of Artificial Sequence: Syntheticpolypeptide

SEQ ID NO: 16 - protein, 108 aa, synthetic construct; identical to SEQ ID NO: 2
  REGION 1..108: note = Description of Artificial Sequence: Syntheticpolypeptide

SEQ ID NO: 17 - protein, 118 aa, synthetic construct
  REGION 1..118: note = Description of Artificial Sequence: Syntheticpolypeptide
EVQLVQSGAEVKKPGASVKVSCKASGYTFTSYGISWVRQAPGQGLEWMGWISAYNGNTNYAQKLQGRVTMTTDTSTSTAYMELRSLRSDDTAVYYCARVGYGGYFDYWGQGTLVTVSS

SEQ ID NO: 18 - protein, 110 aa, synthetic construct
  REGION 1..110: note = Description of Artificial Sequence: Syntheticpolypeptide
SYELMQPPSVSKGLRQTATLTCTGNSNNVGNQGADWLQQHQGHPPKLLSYRNNDRPSGISERFSASRSGSTASLTITGLQPEDEADYYCLAWDSSLSAWVFGGGTKVTVL

SEQ ID NO: 19 - protein, 118 aa, synthetic construct
  REGION 1..118: note = Description of Artificial Sequence: Syntheticpolypeptide
QMQLVQSGAEVKKPGASVTVSCKASGYTFTNSYIHWVRQAPGQGLEWVGRLIPSSGYTIFSQKLQGRVSMTRDTSMSTHYLTLSHLRPEDTAVYYCATDGGNYNLDFWGQGTLVTVSS

SEQ ID NO: 20 - protein, 110 aa, synthetic construct
  REGION 1..110: note = Description of Artificial Sequence: Syntheticpolypeptide
QPVLTQPPSVSGSPGQSVTISCTGTSSDVGGYNYVSWYQQHPGKAPKLMIYDVSSRPSGVSNRFSGSKSDNTASLTISGLQAEDEADYYCSSYTSSSPYVFGTGTKVTVL

SEQ ID NO: 21 - protein, 117 aa, synthetic construct
  REGION 1..117: note = Description of Artificial Sequence: Syntheticpolypeptide
EVQLVQSGTEVKKPGSSVKVSCKASGGSFSNYAISWVRQAPGQGLEWMGRIIPILGIANYAQKFQGRVTITADKSTSTAYMELSSLGSEDTAVYYCARESGSYLDPWGQGTLVTVSS

SEQ ID NO: 22 - protein, 113 aa, synthetic construct
  REGION 1..113: note = Description of Artificial Sequence: Syntheticpolypeptide
DIVMTQSPDSLAVSLGERATINCKSSQSVLYSPNNKNYLTWYQQKPGQPPKLLMYWASTRESGVPDRFSASGSGTDFTLTISSLQAEDVAVYYCQQSRSGPYTFGQGTKVEIK

SEQ ID NO: 23 - protein, 118 aa, synthetic construct
  REGION 1..118: note = Description of Artificial Sequence: Syntheticpolypeptide
EVQLVESGGGFVKPGRSLRLSCTASGFTFGDYGMSWFRQAPGKGLEWVGFIRSKAYGGTTDYAASVKGRFTISRDDSKSFAYLQMNSLKTEDTAVYYCTRGHYSASIWGQGTLVTVSS

SEQ ID NO: 24 - protein, 108 aa, synthetic construct
  REGION 1..108: note = Description of Artificial Sequence: Syntheticpolypeptide
SYELMQPPSVSVAPGKTARITCGGNNIGSKSVHWYQQRPDQAPVLVIYSDNDRPSGIPERFSGSSSGHTATLTISRVEAGDEADYFCQVWDSNKNEWVFGGGTKLTVL

SEQ ID NO: 25 - protein, 123 aa, synthetic construct
  REGION 1..123: note = Description of Artificial Sequence: Syntheticpolypeptide
QVQLVQSGAEVKKPGASVKVSCKASGYAFDGHYMHWVRQAPGQRLEWMGWVDPHSGATNYAQNFQGGVTMTRDTSINTVYMELSSLKSDDTAVYYCARDFYDTSAKSGAFDIWGQGTMVTVSS

SEQ ID NO: 26 - protein, 107 aa, synthetic construct
  REGION 1..107: note = Description of Artificial Sequence: Syntheticpolypeptide
AIQLTQSPSSVSASVGDRVTITCRASQGISSWLAWYQQKPGKAPKLLIYAASSLQSGVPSRFSGSGSGTDFTLTISSLQPEDFATYYCQQVNSFPWAFGQGTKVEIK

SEQ ID NO: 27 - protein, 124 aa, synthetic construct
  REGION 1..124: note = Description of Artificial Sequence: Syntheticpolypeptide
QVQLVQSGAEVKKPGASVKVSCKTSGNTFTNYYMHWVRQAPGQGLEWMGIMNPSGGSTSYAQKFQGRVTMTRDKSTSTVYMELSSLTSEDTAVYYCARDLFPHIYGNYYGMDIWGQGTTVTVSS

SEQ ID NO: 28 - protein, 111 aa, synthetic construct
  REGION 1..111: note = Description of Artificial Sequence: Syntheticpolypeptide
QSVVTQPPSVSAAPGQNVTISCSGSSSNIGNNYVSWYQQLPGTAPKLLIYDNNRRASGIPDRFSGSKSGTSATLGITGLQTGDEADYYCGTWDRSLTTDWVFGGGTKLTVL

SEQ ID NO: 29 - protein, 119 aa, synthetic construct
  REGION 1..119: note = Description of Artificial Sequence: Syntheticpolypeptide
QVQLVESGGGLIQPGGSLRLSCAASGFTVSSAYMSWVRQAPGKGLEWVSVIYRGGTTYYADSVKGRFTISRDNSKNTLYLQMNSLRAEDTAVYYCRGEGGNSGDYFDYWGQGTTVTVSS

SEQ ID NO: 30 - protein, 112 aa, synthetic construct
  REGION 1..112: note = Description of Artificial Sequence: Syntheticpolypeptide
NFMLTQPASVSGSPGQSITISCTGTSSDVGGYNFVSWYQQHPGKAPKLMIYDVSKRPSGVSNRFSGSKSGNTASLTISGLQAEDEADYYCSSYTSTNTLDVLFGGGTKLTVL

SEQ ID NO: 31 - protein, 126 aa, synthetic construct
  REGION 1..126: note = Description of Artificial Sequence: Syntheticpolypeptide
QVQLVQSGAEVKKPGASVKVSCKASGYTFTSYYMHWVRQAPGQGLEWMGIINPSGGSTSYAQKFQGRVTMTRDTSTSTVYMELSGLRSEDTAVYYCARYEHDYDSSKATTGYFDYWGQGTLVTVSS

SEQ ID NO: 32 - protein, 113 aa, synthetic construct
  REGION 1..113: note = Description of Artificial Sequence: Syntheticpolypeptide
AIQLTQSPDSLAVSLGERATINCKSSQSILYRSNNKNYLAWYQQKPGQPPKLLIYWASTRESGVPDRFSGSGSGTDFTLTISSLQPEDFATYYCQQADRFPITFGQGTRLEIK

SEQ ID NO: 33 - protein, 121 aa, synthetic construct
  REGION 1..121: note = Description of Artificial Sequence: Syntheticpolypeptide
QVQLQQSGPGLVKPSQTLSLTCAISGDSVSSNSAAWNWIRQSPSRGLEWLGRTYYRSKWYNDYAVSVKSRITINPDTSKNQFSLQLNSVTPEDTAVYYCARDRWELPFDYWGQGTTVTVSS

SEQ ID NO: 34 - protein, 110 aa, synthetic construct
  REGION 1..110: note = Description of Artificial Sequence: Syntheticpolypeptide
QSVVTQPPSVSAASGQKVIISCSGSNSNIVNNYVSWYQQLPGAAPKVLIYANNKRPSGIPDRFSGSKSGTSAFLAITGLQTGDEADYYCGTWDGSLDVDVFGGGTKLTVL

SEQ ID NO: 35 - protein, 121 aa, synthetic construct
  REGION 1..121: note = Description of Artificial Sequence: Syntheticpolypeptide
EVQLVESGAEVKKPGASVKVSCKASGYTFTSYGISWVRQAPGQGLEWMGWISAYNGNTNYAQKLQGRVTMTTDTSTSTAYMELRSLRSDDTAVYYCARGPGILTGYYFDYWGQGTLVTVSS

SEQ ID NO: 36 - protein, 107 aa, synthetic construct
  REGION 1..107: note = Description of Artificial Sequence: Syntheticpolypeptide
EIVMTQSPSSLSASVGDRVTITCRASQGINYHLAWYQQKPGKAPKLLIYAASALQSGVPSRFSGTGSGTEFTLTISSLQPEDFATYYCQQFNTYPLTFGGGTKLEIK

SEQ ID NO: 37 - protein, 123 aa, synthetic construct
  REGION 1..123: note = Description of Artificial Sequence: Syntheticpolypeptide
QVQLQQSGPGLVKPSQTLSLTCAISGDSVSSNSAAWNWIRQSPSRGLEWLGRTYYRSKWYNDYAVSVKSRITINPDTSKNQFSLQLNSVTPEDTAVYYCAMHSGYRNYGMDVWGQGTTVTVSS

SEQ ID NO: 38 - protein, 112 aa, synthetic construct
  REGION 1..112: note = Description of Artificial Sequence: Syntheticpolypeptide
QSVVTQPPSVSGAPGQRVTISCTGSSSNIGAGYDVHWYQQLPGTAPKLLIYGNSNRPSGVPDRFSGSKSGTSASLAITGLQAEDEADYYCQSYDSSLSGAVVFGGGTKLTVL

SEQ ID NO: 39 - protein, 125 aa, synthetic construct; identical to SEQ ID NO: 11
  REGION 1..125: note = Description of Artificial Sequence: Syntheticpolypeptide

SEQ ID NO: 40 - protein, 110 aa, synthetic construct
  REGION 1..110: note = Description of Artificial Sequence: Syntheticpolypeptide
SYELMQPPSTSGTPGQRVTISCSGSSSNIGSHIVNGYQQFPGAAPQLLIYNDDQRPSGVPDRFSGSKSGASASLAISGLQSEDEAHYYCSAWDDILKGPVFGGGTKVTVL

SEQ ID NO: 41 - protein, 121 aa, synthetic construct
  REGION 1..121: note = Description of Artificial Sequence: Syntheticpolypeptide
QVQLVQSGAEVKKPGASVKVSCEASGYTFTNYYIHWLRQAPGQGLEWMGIINPSGGSTTYAQKFQGRITMTRDTSTNTLYMELSSLRSEDTAIYYCARRDCRGPSCYFAYWGQGTTVTVSS

SEQ ID NO: 42 - protein, 107 aa, synthetic construct
  REGION 1..107: note = Description of Artificial Sequence: Syntheticpolypeptide
DIVMTQSPSSLSASVGDRVTITCRASQSISSYLNWYQQKPGKAPKLLIYAASSLQSGVPPRFSGSGSGTEFTLTISSLQPEDFATYYCQQANSFPPTFGQGTKVDIK

SEQ ID NO: 43 - protein, 114 aa, synthetic construct
  REGION 1..114: note = Description of Artificial Sequence: Syntheticpolypeptide
EVQLVESGGGLVQPGRSLRLSCRGSNFNFDDLAISWVRQAPGKGLEWLGFVRSKAYGETTDYVASVKGRFTISRDDSKFIAWLQMDSLKTDDTAVYYCTTFNYWGQGTLVTVSS

SEQ ID NO: 44 - protein, 108 aa, synthetic construct
  REGION 1..108: note = Description of Artificial Sequence: Syntheticpolypeptide
QPVLTQPPSVSVAPGKTARISCGGNNIASEAVHWYQKKPGQAPVLVIYYDSDRPSGIPERFSGSNSGNTATLRISRVDAGDEADYYCQVWDRTTDQPVFGGGTKLTVL

SEQ ID NO: 45 - protein, 4 aa, unidentified
  REGION 1..4: note = Description of Unknown:Hinge region sequence
CPSC

SEQ ID NO: 46 - protein, 4 aa, unidentified
  REGION 1..4: note = Description of Unknown:Hinge region sequence
CPPC